European Patent Application EP 4 545 640 A1, published April 30, 2025. Title: A combination of a Livin inhibitor and an inhibitor of the interaction between PD-1 and its ligand PD-L1 or their intracellular downstream signaling pathways. Applicant: King Faisal Specialist Hospital & Research Centre, Riyadh. The sequence listing filed with the application follows.

SEQUENCE LISTING (18 sequences)

SEQ ID NO: 1 - DNA, 21 bp, synthetic construct
  misc_feature 1..19: note = RNA
  misc_feature 20..21: note = DNA
  source 1..21: mol_type = other DNA
  modified_base 1..19: mod_base = OTHER; note = uracil
ggcatttgctgaacgcatttt

SEQ ID NO: 2 - RNA, 21 nt, synthetic construct
  source 1..21: mol_type = other RNA
aatgcgttcagcaaatgccag

SEQ ID NO: 3 - DNA, 21 bp, synthetic construct
  misc_feature 1..19: note = RNA
  misc_feature 20..21: note = DNA
  source 1..21: mol_type = other DNA
  modified_base 1..19: mod_base = OTHER; note = uracil
tatacatagtgtgatttgctt

SEQ ID NO: 4 - DNA, 21 bp, synthetic construct
  misc_feature 1..19: note = RNA
  misc_feature 20..21: note = DNA
  source 1..21: mol_type = other DNA
  modified_base 1..19: mod_base = OTHER; note = uracil
gcaaatcacactatgtatatt

SEQ ID NO: 5 - DNA, 21 bp, synthetic construct
  misc_feature 1..19: note = RNA
  misc_feature 20..21: note = DNA
  source 1..21: mol_type = other DNA
  modified_base 1..19: mod_base = OTHER; note = uracil
ggaagagactttgtccacatt

SEQ ID NO: 6 - DNA, 21 bp, synthetic construct
  misc_feature 1..19: note = RNA
  misc_feature 20..21: note = DNA
  source 1..21: mol_type = other DNA
  modified_base 1..19: mod_base = OTHER; note = uracil
tgtggacaaagtctcttcctt

SEQ ID NO: 7 - DNA, 21 bp, synthetic construct
  misc_feature 1..19: note = RNA
  misc_feature 20..21: note = DNA
  source 1..21: mol_type = other DNA
  modified_base 1..19: mod_base = OTHER; note = uracil
tttatttatgattaaatcctt

SEQ ID NO: 8 - DNA, 21 bp, synthetic construct
  misc_feature 1..19: note = RNA
  misc_feature 20..21: note = DNA
  source 1..21: mol_type = other DNA
  modified_base 1..19: mod_base = OTHER; note = uracil
ggatttaatcataaataaatt

SEQ ID NO: 9 - DNA, 21 bp, synthetic construct
  misc_feature 1..19: note = RNA
  misc_feature 20..21: note = DNA
  source 1..21: mol_type = other DNA
  modified_base 1..19: mod_base = OTHER; note = uracil
taaatttaacacattctgctt

SEQ ID NO: 10 - DNA, 21 bp, synthetic construct
  misc_feature 1..19: note = RNA
  misc_feature 20..21: note = DNA
  source 1..21: mol_type = other DNA
  modified_base 1..19: mod_base = OTHER; note = uracil
gcagaatgtgttaaatttatt

SEQ ID NO: 11 - DNA, 21 bp, synthetic construct
  misc_feature 1..19: note = RNA
  misc_feature 20..21: note = DNA
  source 1..21: mol_type = other DNA
  modified_base 1..19: mod_base = OTHER; note = uracil
tatatatatatatatatgctt

SEQ ID NO: 12 - DNA, 21 bp, synthetic construct
  misc_feature 1..19: note = RNA
  misc_feature 20..21: note = DNA
  source 1..21: mol_type = other DNA
  modified_base 1..19: mod_base = OTHER; note = uracil
gcatatatatatatatatatt

SEQ ID NO: 13 - DNA, 21 bp, synthetic construct
  misc_feature 1..19: note = RNA
  misc_feature 20..21: note = DNA
  source 1..21: mol_type = other DNA
  modified_base 1..19: mod_base = OTHER; note = uracil
ttaatacaacgtttaatcctt

SEQ ID NO: 14 - DNA, 21 bp, synthetic construct
  misc_feature 1..19: note = RNA
  misc_feature 20..21: note = DNA
  source 1..21: mol_type = other DNA
  modified_base 1..19: mod_base = OTHER; note = uracil
ggattaaacgttgtattaatt

SEQ ID NO: 15 - DNA, 21 bp, synthetic construct
  misc_feature 1..19: note = RNA
  misc_feature 20..21: note = DNA
  source 1..21: mol_type = other DNA
  modified_base 1..19: mod_base = OTHER; note = uracil
tttgaattcgtatccatcctt

SEQ ID NO: 16 - DNA, 21 bp, synthetic construct
  misc_feature 1..19: note = RNA
  misc_feature 20..21: note = DNA
  source 1..21: mol_type = other DNA
  modified_base 1..19: mod_base = OTHER; note = uracil
ggatggatacgaattcaaatt

SEQ ID NO: 17 - DNA, 21 bp, synthetic construct
  misc_feature 1..19: note = RNA
  misc_feature 20..21: note = DNA
  source 1..21: mol_type = other DNA
  modified_base 1..19: mod_base = OTHER; note = uracil
ttatatatggatagtttcctt

SEQ ID NO: 18 - DNA, 21 bp, synthetic construct
  misc_feature 1..19: note = RNA
  misc_feature 20..21: note = DNA
  source 1..21: mol_type = other DNA
  modified_base 1..19: mod_base = OTHER; note = uracil
ggaaactatccatatataatt